European Patent Application EP 4 803 624 A1, published September 9, 2026. Title: ＢＣＬ１１Ａ遺伝子のエンハンサーの一部又は全部が破壊された造血幹細胞の製造方法、及びその方法に用いるためのキット. Applicant: C4U Corporation. The sequence listing filed with the application follows.

SEQUENCE LISTING (27 sequences)

SEQ ID NO: 1 - protein, 887 aa, Escherichia coli
  source 1..887: note = cas3
EPFKYICHYWGKSSKSLTKGNDIHLLIYHCLDVAAVADCWWDQSVVLQNTFCRNEMLSKQRVKAWLLFFIALHDIGKFDIRFQYKSAESWLKLNPATPSLNGPSTQMCRKFNHGAAGLYWFNQDSLSEQSLGDFFSFFDAAPHPYESWFPWVEAVTGHHGFILHSQDQDKSRWEMPASLASYAAQDKQAREEWISVLEALFLTPAGLSINDIPPDCSSLLAGFCSLADWLGSWTTTNTFLFNEDAPSDINALRTYFQDRQQDASRVLELSGLVSNKRCYEGVHALLDNGYQPRQLQVLVDALPVAPGLTVIEAPTGSGKTETALAYAWKLIDQQIADSVIFALPTQATANAMLTRMEASASHLFSSPNLILAHGNSRFNHLFQSIKSRAITEQGQEEAWVQCCQWLSQSNKKVFLGQIGVCTIDQVLISVLPVKHRFIRGLGIGRSVLIVDEVHAYDTYMNGLLEAVLKAQADVGGSVILLSATLPMKQKQKLLDTYGLHTDPVENNSAYPLINWRGVNGAQRFDLLAHPEQLPPRFSIQPEPICLADMLPDLTMLERMIAAANAGAQVCLICNLVDVAQVCYQRLKELNNTQVDIDLFHARFTLNDRREKENRVISNFGKNGKRNVGRILVATQVVEQSLDVDFDWLITQHCPADLLFQRLGRLHRHHRKYRPAGFEIPVATILLPDGEGYGRHEHIYSNVRVMWRTQQHIEELNGASLFFPDAYRQWLDSIYDDAEMDEPEWVGNGMDKFESAECEKRFKARKVLQWAEEYSLQDNDETILAVTRDGEMSLPLLPYVQTSSGKQLLDGQVYEDLSHEQQYEALALNRVNVPFTWKRSFSEVVDEDGLLWLEGKQNLDGWVWQGNSIVITYTGDEGMTRVIPANPK

SEQ ID NO: 2 - DNA, 2661 bp, Escherichia coli
  source 1..2661: mol_type = genomic DNA; note = cas3
gaacccttcaagtacatctgccactactggggcaagagcagcaagagcctgaccaagggcaacgacatccatctgctgatctaccactgcctggatgtggccgctgtggctgactgttggtgggatcagtctgtggtgctgcagaacaccttctgccggaacgagatgctgagcaagcagagagtgaaggcctggctgctgttctttatcgccctgcacgacatcggcaagttcgacatccggttccagtacaagagcgccgagagctggctgaagctgaaccctgctacacccagcctgaacggccctagcacacagatgtgccggaagttcaatcacggcgctgccggcctgtactggttcaaccaggatagcctgagcgagcagtccctgggcgacttcttcagcttcttcgacgccgctcctcatccttacgagtcctggtttccttgggtcgaagccgtgacaggccaccacggctttattctgcacagccaggaccaggacaagagcagatgggagatgcctgccagcctggcctcttatgccgctcaggataagcaggcccgggaagagtggatctctgtgctggaagccctgtttctgacaccagccggcctgagcatcaacgatatccctccagattgcagcagcctgctggccggcttttgttctctggccgattggctcggcagctggacaaccaccaacacctttctgttcaacgaggacgcccctagcgacatcaacgccctgagaacctacttccaggacagacagcaggacgccagcagagtgctggaactgtctggcctggtgtccaacaagagatgctacgaaggggtgcacgccctgctggacaatggctatcagcctagacagctgcaggtcctggtggatgctctgcctgttgctcctggcctgacagtgattgaagcccctacaggcagcggcaagacagaaacagccctggcctatgcctggaagctgatcgaccagcagatcgccgacagcgtgatcttcgctctgccaacacaggccacagccaacgccatgctgaccagaatggaagcctctgccagccacctgttcagcagccccaatctgattctggcccacggcaacagcagattcaatcacctgttccagagcatcaagtcccgggccatcacagagcagggacaagaggaagcttgggtgcagtgctgtcagtggctgagccagagcaacaagaaagtgttcctgggccagatcggcgtgtgcaccattgaccaggtgctgatctcagtgctgcccgtgaagcaccggttcatcagaggactcggcatcggcagatccgtgctgatcgtggatgaagtgcacgcctacgacacctacatgaacggcctgcttgaggccgtgctgaaagcccaggctgatgttggcggaagcgtgatcctgctgagcgccacactgcctatgaagcagaagcagaaactgctggatacctacggcctgcacaccgatcctgtggaaaacaacagcgcctatcctctgatcaattggagaggcgtgaacggcgcccagagattcgatctgcttgcccatcctgagcagctgcctccaagattcagcatccagcctgagcctatctgcctggccgacatgctgcctgacctgaccatgctggaacggatgatcgccgctgctaatgccggtgctcaagtgtgcctgatctgcaacctggtggacgtggcccaagtgtgctaccagagactgaaagagctgaacaacacccaggtggacatcgacctgtttcacgcccggttcaccctgaacgaccggcgcgagaaagaaaacagagtgatcagcaacttcggcaagaacggcaagcggaatgtgggcagaatcctggtggctacacaggtggtggaacagagcctggacgtggacttcgactggctgatcacccagcactgtcccgccgacctgctgtttcaaagactgggcagactgcaccggcaccaccggaagtatagacctgccggctttgagatccccgtggccacaattttgctgcccgatggcgaaggctacggcagacacgagcacatctacagcaacgtgcgagtgatgtggcggacccagcagcacatcgaggaactgaatggcgccagcctgttcttccctgatgcctatcgacagtggctggacagcatctacgacgacgccgagatggatgagcctgagtgggtcggaaacggcatggacaagtttgagtccgccgagtgcgagaagcggttcaaggccagaaaggttctgcagtgggccgaagagtacagcctgcaggacaacgacgagacaatcctggccgtgaccagagatggcgagatgtctctgcctctgctgccctacgtgcagaccagctctggaaaacagctgctggacggccaggtgtacgaggatctgtctcacgagcagcagtacgaggccctggctctgaatagagtgaacgtgcccttcacctggaagcggagctttagcgaagtggtggacgaggatggactgctgtggctcgaagggaagcagaatctggacggctgggtctggcagggcaactccatcgtgatcacctacacaggcgacgagggcatgacaagagtgatccccgccaatcctaag

SEQ ID NO: 3 - protein, 501 aa, Escherichia coli
  source 1..501: note = cse1
NLLIDNWIPVRPRNGGKVQIINLQSLYCSRDQWRLSLPRDDMELAALALLVCIGQIIAPAKDDVEFRHRIMNPLTEDEFQQLIAPWIDMFYLNHAEHPFMQTKGVKANDVTPMEKLLAGVSGATNCAFVNQPGQGEALCGGCTAIALFNQANQAPGFGGGFKSGLRGGTPVTTFVRGIDLRSTVLLNVLTLPRLQKQFPNESHTENQPTWIKPIKSNESIPASSIGFVRGLFWQPAHIELCDPIGIGKCSCCGQESNLRYTGFLKEKFTFTVNGLWPHPHSPCLVTVKKGEVEEKFLAFTTSAPSWTQISRVVVDKIIQNENGNRVAAVVNQFRNIAPQSPLELIMGGYRNNQASILERRHDVLMFNQGWQQYGNVINEIVTVGLGYKTALRKALYTFAEGFKNKDFKGAGVSVHETAERHFYRQSELLIPDVLANVNFSQADEVIADLRDKLHQLCEMLFNQSVAPYAHHPKLISTLALARATLYKHLRELKPQGGPSNG

SEQ ID NO: 4 - DNA, 1503 bp, Escherichia coli
  source 1..1503: mol_type = genomic DNA; note = cse1
aacctgctgatcgacaactggatccccgtgcggcctagaaatggcggcaaggtgcagatcatcaatctgcagagcctgtactgcagccgggatcagtggcgactgagcctgcctagagatgacatggaactggccgctctggctctgctcgtgtgcatcggacagattatcgcccctgccaaggatgatgtggaattccggcacagaatcatgaaccctctgaccgaggacgagttccagcagctgatcgccccttggatcgacatgttctacctgaaccacgccgagcatcccttcatgcagaccaagggcgtgaaagccaacgatgtgacccctatggaaaaactgctggccggcgtttccggcgccacaaactgtgcctttgtgaaccagcctggacagggcgaagctctgtgtggcggatgtacagcaatcgccctgttcaaccaggccaatcaggcccctggattcggcggaggctttaagtctggactgagaggcggaacccctgtgaccacatttgtgcggggcatcgacctgagaagcaccgtgctgctgaacgtcctgacactgcccagactgcagaagcagttccccaacgagagccacaccgagaaccagccaacctggatcaagcccatcaagagcaacgagtctatccccgccagctccatcggctttgtcagaggcctgttttggcagcccgctcacatcgagctgtgcgaccctatcggcatcggcaagtgtagctgttgcggccaagagtccaacctgcggtacaccggctttctgaaagagaagttcaccttcaccgtgaacggcttgtggccccatccacacagcccttgtctcgtgaccgtgaagaaaggcgaggtcgaggaaaagttcctggcctttaccacaagcgcccctagctggacccagatctctagagtggtggtggacaagatcatccagaacgagaacggcaatagagtggccgccgtggtcaaccagttccggaatattgcccctcagagccctctggaactgatcatgggcggctaccggaacaaccaggctagcatcctggaaagacggcacgatgtgctgatgttcaatcaaggatggcagcagtacggcaacgtgatcaacgagatcgtgacagtcggcctgggctacaagacagccctgagaaaggccctgtacaccttcgccgagggcttcaagaacaaggacttcaaaggcgcaggcgtgtccgtgcacgaaacagccgagagacacttctaccggcagagcgagctgctgattcctgacgtgctggccaacgtgaacttcagccaggccgatgaagtgatcgccgacctgagggacaaactgcatcagctgtgtgaaatgctgtttaaccagagcgtggccccttacgctcatcaccccaagctgattagcactctggccctggctagagctaccctgtacaagcacctgagagagctgaagcctcaaggcggccctagcaatgga

SEQ ID NO: 5 - protein, 159 aa, Escherichia coli
  source 1..159: note = cse2
ADEIDAMALYRAWQQLDNGSCAQIRRVSEPDELRDIPAFYRLVQPFGWENPRHQQALLRMVFCLSAGKNVIRHQDKKSEQTTGISLGRALANSGRINERRIFQLIRADRTADMVQLRRLLTHAEPVLDWPLMARMLTWWGKRERQQLLEDFVLTTNKNA

SEQ ID NO: 6 - DNA, 477 bp, Escherichia coli
  source 1..477: mol_type = genomic DNA; note = cse2
gccgacgagatcgacgccatggcactgtatagagcctggcagcagctggacaatggcagctgtgcccagatcagaagagtgtccgagcctgacgagctgagagacatccccgccttctacagactggtgcagcctttcggctgggagaaccctagacatcagcaggcactgctgcggatggtgttctgtctgagcgccggcaagaacgtgatccggcaccaggataagaagtccgagcagaccacaggcatcagcctgggtagagccctggccaatagcggcagaatcaacgagcggcggatcttccagctgatcagagccgatagaaccgccgatatggtgcagctcagacggctgctgacacacgctgaacctgtgctggattggcccctgatggccagaatgctgacttggtggggaaagagagagcgccagcagctcctggaagatttcgtgctgaccaccaacaagaacgcc

SEQ ID NO: 7 - protein, 223 aa, Escherichia coli
  source 1..223: note = cas5
RSYLILRLAGPMQAWGQPTFEGTRPTGRFPTRSGLLGLLGACLGIQRDDTSSLQALSESVQFAVRCDELILDDRRVSVTGLRDYHTVLGAREDYRGLKSHETIQTWREYLCDASFTVALWLTPHATMVISELEKAVLKPRYTPYLGRRSCPLTHPLFLGTCQASDPQKALLNYEPVGGDIYSEESVTGHHLKFTARDEPMITLPRQFASREWYVIKGGMDVSQ

SEQ ID NO: 8 - DNA, 669 bp, Escherichia coli
  source 1..669: mol_type = genomic DNA; note = cas5
cgcagctacctgatcctgagactggccggacctatgcaggcttggggacagcctaccttcgagggcacaagacccaccggcagattccctacaagaagcggcctgctgggactgcttggagcctgtctgggaatccagagggacgatacaagctccctgcaggctctgagcgagagcgtgcagtttgccgtcagatgcgacgaactgatcctggatgacagacgggtgtccgtgaccggcctgagagattaccatacagtgctgggcgccagagaggattaccggggactgaaaagccacgaaaccatccagacctggcgcgagtacctgtgcgacgcctcttttacagtggccctgtggctgacacctcacgccacaatggtcatctctgagctggaaaaggccgtgctgaagccccggtacacaccttacctgggcagaagaagctgccctctgacacaccctctgtttctgggcacctgtcaggccagcgatccacagaaagctctgctgaactacgagcctgtcggcggcgacatctacagcgaggaatctgtgacaggccaccacctgaagtttaccgccagagatgagcctatgatcaccctgcctcggcagttcgcctccagagagtggtacgttatcaaaggcggcatggatgtgtcccag

SEQ ID NO: 9 - protein, 198 aa, Escherichia coli
  source 1..198: note = cas6
YLSKVIIARAWSRDLYQLHQGLWHLFPNRPDAARDFLFHVEKRNTPEGCHVLLQSAQMPVSTAVATVIKTKQVEFQLQVGVPLYFRLRANPIKTILDNQKRLDSKGNIKRCRVPLIKEAEQIAWLQRKLGNAARVEDVHPISERPQYFSGDGKSGKIQTVCFEGVLTINDAPALIDLVQQGIGPAKSMGCGLLSLAPL

SEQ ID NO: 10 - DNA, 594 bp, Escherichia coli
  source 1..594: mol_type = genomic DNA; note = cas6
tacctcagcaaagtgatcattgccagagcttggagcagggacctgtaccagctgcatcaaggcctgtggcatctgttccccaatagacccgacgccgccagggatttcctgtttcacgtggaaaagcggaacacccctgagggctgtcatgtgctgctgcagagtgctcagatgccagtgtcaactgccgtggccaccgtgatcaagaccaagcaggtcgaattccagctccaagtgggcgtgcccctgtacttcagactgagagccaatcctatcaagacgatcctggacaaccagaagcggctggacagcaagggcaacatcaagagatgcagggtgcccctgatcaaagaggccgaacagattgcctggctgcagcggaaactgggaaatgccgccagagtggaagatgtgcaccccatcagcgagcggcctcagtactttagcggagatggcaagtccggcaagatccagaccgtgtgctttgagggcgtgctgacaatcaacgacgcccctgctctgatcgacctggtccagcaaggcattggcccagccaagtctatgggctgtggactgctgtctctggcccctctg

SEQ ID NO: 11 - protein, 362 aa, Escherichia coli
  source 1..362: note = cas7
SNFINIHVLISHSPSCLNRDDMNMQKDAIFGGKRRVRISSQSLKRAMRKSGYYAQNIGESSLRTIHLAQLRDVLRQKLGERFDQKIIDKTLALLSGKSVDEAEKISADAVTPWVVGEIAWFCEQVAKAEADNLDDKKLLKVLKEDIAAIRVNLQQGVDIALSGRMATSGMMTELGKVDGAMSIAHAITTHQVDSDIDWFTAVDDLQEQGSAHLGTQEFSSGVFYRYANINLAQLQENLGGASREQALEIATHVVHMLATEVPGAKQRTYAAFNPADMVMVNFSDMPLSMANAFEKAVKAKDGFLQPSIQAFNQYWDRVANGYGLNGAAAQFSLSDVDPITAQVKQMPTLEQLKSWVRNNGEA

SEQ ID NO: 12 - DNA, 1086 bp, Escherichia coli
  source 1..1086: mol_type = genomic DNA; note = cas7
tccaacttcatcaacatccacgtgctgatctctcacagccccagctgcctgaaccgggacgacatgaacatgcagaaggacgccatcttcggcggcaagagaagagtgcggatcagcagccagagcctgaagcgggccatgagaaagagcggctactacgcccagaacatcggcgagagcagcctgagaacaatccatctggcccagctgcgggacgtgctgagacagaaactgggcgagagattcgaccagaagatcatcgacaagacactggccctgctgagcggcaagtctgtggatgaggccgagaagatcagcgccgatgctgtgacaccttgggtcgtgggagagatcgcctggttctgtgaacaggtggccaaggccgaggccgacaacctggacgataagaaactgctgaaggtgctgaaagaggatatcgccgccatcagagtgaacctgcagcagggcgttgacattgccctgtctggcagaatggccaccagcggcatgatgaccgagctgggaaaagtggacggcgccatgtctatcgcccacgccattacaacacaccaggtggacagcgacatcgactggttcaccgccgtggacgatctgcaagaacagggatctgcccacctgggcacccaagagtttagcagcggcgtgttctacagatacgccaacatcaacctggctcagctgcaagagaatctcggcggagcctctagagagcaggccctggaaattgccacacacgtggtgcacatgctggccacagaagtgcctggcgccaagcagagaacctacgccgcctttaatcccgccgacatggtcatggtcaacttcagcgacatgcccctgagcatggccaacgcctttgagaaggccgtgaaggccaaggacggcttcctgcagcctagcatccaggccttcaatcagtactgggacagagtggccaacggctacggactgaatggtgccgccgctcagtttagcctgtccgacgtggaccctatcacagcccaagtgaagcagatgcccacactggaacagctgaagtcctgggtccgaaacaacggcgaggcc

SEQ ID NO: 13 - DNA, 35 bp, Homo sapiens
  source 1..35: mol_type = genomic DNA; note = crRNA-target
aagtcctgtctagctgccttccttatcacaggaat

SEQ ID NO: 14 - DNA, 23 bp, Homo sapiens
  source 1..23: mol_type = genomic DNA; note = gRNA-target
ctaacagttgcttttatcacagg

SEQ ID NO: 15 - DNA, 22 bp, synthetic construct
  source 1..22: mol_type = other DNA; note = Target probe
ttatcacaggctccaggaaggg

SEQ ID NO: 16 - DNA, 20 bp, synthetic construct
  source 1..20: mol_type = other DNA; note = Target Fwd
tgattccagtgcaaagtcca

SEQ ID NO: 17 - DNA, 20 bp, synthetic construct
  source 1..20: mol_type = other DNA; note = Target Rev
caccctaatcagaggccaaa

SEQ ID NO: 18 - DNA, 24 bp, synthetic construct
  source 1..24: mol_type = other DNA; note = Reference probe
tagatgtggcaagtcagaccacag

SEQ ID NO: 19 - DNA, 20 bp, synthetic construct
  source 1..20: mol_type = other DNA; note = Reference Fwd
tgaagttttccaggggtttg

SEQ ID NO: 20 - DNA, 20 bp, synthetic construct
  source 1..20: mol_type = other DNA; note = Reference Rev
ctttctctgagggcatggag

SEQ ID NO: 21 - DNA, 19 bp, synthetic construct
  source 1..19: mol_type = other DNA; note = g globin Fwd
cttccttgggagatgccat

SEQ ID NO: 22 - DNA, 21 bp, synthetic construct
  source 1..21: mol_type = other DNA; note = g globin Rev
gaattctttgccgaaatggat

SEQ ID NO: 23 - DNA, 19 bp, synthetic construct
  source 1..19: mol_type = other DNA; note = b globin Fwd
ctttagtgatggcctggct

SEQ ID NO: 24 - DNA, 19 bp, synthetic construct
  source 1..19: mol_type = other DNA; note = b globin Rev
cactggtggggtgaattct

SEQ ID NO: 25 - DNA, 22 bp, synthetic construct
  source 1..22: mol_type = other DNA; note = ACTB Fwd
caccattggcaatgagcggttc

SEQ ID NO: 26 - DNA, 22 bp, synthetic construct
  source 1..22: mol_type = other DNA; note = ACTB Rev
aggtctttgcggatgtccacgt

SEQ ID NO: 27 - RNA, 32 nt, synthetic construct
  source 1..32: mol_type = other RNA; note = crRNA
attcctgtgataaggaaggcagctagacagga